European Patent Application EP 4 393 943 A1, published July 3, 2024. Title: POLYPEPTIDE FUSION MOLECULE CLOSE TO NATURAL MOLECULE. Applicant: TIOC THERAPEUTICS, LTD. The sequence listing filed with the application follows.

SEQUENCE LISTING (38 sequences)

SEQ ID NO: 1 - protein, 200 aa, synthetic construct
  source 1..200: note = Amino acid sequence of 1G4 TCR alpha chain with mutation
AQEVTQIPAALSVPEGENLVLNCSFTDSAIYNLQWFRQDPGKGLTSLLLITPWQREQTSGRLNASLDKSSGRSTLYIAASQPGDSATYLCAVRPLVDPTYIPTFGRGTSLIVHPYIQNPDPAVYQLRDSKSSDKSVCLFTDFDSQTNVSQSKDSDVYITDKCVLDMRSMDFKSNSAVAWSNKSDFACANAFNNSIIPEDT

SEQ ID NO: 2 - DNA, 600 bp, synthetic construct
  source 1..600: mol_type = other DNA; note = Nucleic acid sequence of 1G4 TCR alpha chain with mutation
gcccaagaagttacccaaatcccggcagccctgagtgtcccggaaggtgaaaatctggtcctgaattgctcgtttaccgatagcgccatttacaacctgcagtggtttcgtcaagatccgggcaaaggtctgaccagcctgctgctgatcacgccgtggcagcgtgaacaaaccagcggccgcctgaatgcctctctggataaaagctctggtcgcagcaccctgtatattgcagcatcacagccgggtgactcggctacgtacctgtgtgcggtgcgtccgctggttgatccgacctatatcccgacgtttggccgcggtaccagtctgattgttcatccgtatatccagaacccggatccggcggtctaccaactgcgtgatagtaaaagttccgacaaatccgtgtgcctgtttaccgatttcgactcacagacgaatgtttcacaatcgaaagattcggacgtctatattaccgataaatgtgtgctggacatgcgcagcatggatttcaaaagcaactctgcagtcgcttggagtaataaatccgactttgcgtgcgccaacgcattcaacaattctattatcccggaagatacg

SEQ ID NO: 3 - protein, 241 aa, synthetic construct
  source 1..241: note = Amino acid sequence of 1G4 TCR beta chain with mutation
GVTQTPKFQVLKTGQSMTLQCAQDMNHEYMSWYRQDPGMGLRLIHYSVAIQTTDQGEVPNGYNVSRSTTEDFPLRLLSAAPSQTSVYFCASSYVGNTGELFFGEGSRLTVLEDLKNVFPPEVAVFEPSEAEISHTQKATLVCLATGFYPDHVELSWWVNGKEVHSGVCTDPQPLKEQPALNDSRYALSSRLRVSATFWQDPRNHFRCQVQFYGLSENDEWTQDRAKPVTQIVSAEAWGRAD

SEQ ID NO: 4 - DNA, 723 bp, synthetic construct
  source 1..723: mol_type = other DNA; note = Nucleic acid sequence of 1G4 TCR beta chain with mutation
ggtgttacccagacgccgaaattccaagtcctgaaaaccggccagtcgatgacgctgcagtgtgcacaagatatgaatcatgaatatatgagctggtaccgccaagacccgggtatgggcctgcgtctgattcactatagcgtggccatccagaccacggatcaaggtgaagttccgaacggctacaatgtctcccgctcaaccacggaagactttccgctgcgtctgctgagcgcagcaccgtcgcagaccagcgtgtatttctgcgcaagctcttacgttggtaacaccggcgaactgtttttcggtgaaggcagccgcctgacggtcctggaagatctgaaaaatgtgtttccgccggaagtcgcggtgttcgaaccgtccgaagccgaaatttcacatacccagaaagcaacgctggtgtgcctggctaccggtttttatccggatcatgtggaactgtcttggtgggttaacggtaaagaagtgcacagtggcgtttgtacggatccgcagccgctgaaagaacaaccggcactgaatgactcccgttatgctctgagttcccgtctgcgcgtttcagccaccttctggcaggatccgcgtaaccactttcgctgtcaggtccaattctacggtctgtctgaaaatgatgaatggacccaggaccgtgcaaaaccggtcacgcaaatcgtgagtgcagaagcttggggccgtgcagat

SEQ ID NO: 5 - protein, 122 aa, Homo sapiens [sequence omitted]

SEQ ID NO: 6 - DNA, 366 bp, Homo sapiens
  source 1..366: mol_type = other DNA
gaagttcagctggtcgaaagcggtggcggtctggtccaaccgggcggttcactgcgtctgtcgtgtgcggcctctggttatagttttaccggctacacgatgaattgggttcgccaggcaccgggtaaaggcctggaatgggtcgctctgattaacccgtataaaggcgtgtctacctacaatcagaaatttaaagatcgcttcaccatcagcgtggacaaatctaaaaacacggcatatctgcaaatgaatagtctgcgtgcagaagataccgctgtgtattactgcgctcgctctggttattacggcgatagtgactggtattttgacgtttggggtcagggcaccctggtgaccgttagttcc

SEQ ID NO: 7 - protein, 370 aa, synthetic construct
  source 1..370: note = Amino acid sequence of fusion protein
EVQLVESGGGLVQPGGSLRLSCAASGYSFTGYTMNWVRQAPGKGLEWVALINPYKGVSTYNQKFKDRFTISVDKSKNTAYLQMNSLRAEDTAVYYCARSGYYGDSDWYFDVWGQGTLVTVSSGGGGSNAGVTQTPKFQVLKTGQSMTLQCAQDMNHEYMSWYRQDPGMGLRLIHYSVAIQTTDQGEVPNGYNVSRSTTEDFPLRLLSAAPSQTSVYFCASSYVGNTGELFFGEGSRLTVLEDLKNVFPPEVAVFEPSEAEISHTQKATLVCLATGFYPDHVELSWWVNGKEVHSGVCTDPQPLKEQPALNDSRYALSSRLRVSATFWQDPRNHFRCQVQFYGLSENDEWTQDRAKPVTQIVSAEAWGRAD

SEQ ID NO: 8 - DNA, 1110 bp, synthetic construct
  source 1..1110: mol_type = other DNA; note = Nucleic acid sequence of fusion protein
gaagttcagctggtcgaaagcggtggcggtctggtccaaccgggcggttcactgcgtctgtcgtgtgcggcctctggttatagttttaccggctacacgatgaattgggttcgccaggcaccgggtaaaggcctggaatgggtcgctctgattaacccgtataaaggcgtgtctacctacaatcagaaatttaaagatcgcttcaccatcagcgtggacaaatctaaaaacacggcatatctgcaaatgaatagtctgcgtgcagaagataccgctgtgtattactgcgctcgctctggttattacggcgatagtgactggtattttgacgtttggggtcagggcaccctggtgaccgttagttccggcggtggcggtagcaacgcaggtgttacccagacgccgaaattccaagtcctgaaaaccggccagtctatgacgctgcagtgtgcgcaagatatgaaccatgaatacatgagttggtaccgtcaggacccgggtatgggtctgcgtctgattcactattctgtggcgatccagaccacggatcaaggtgaagttccgaacggctacaatgtctcgcgtagcaccacggaagactttccgctgcgtctgctgtccgcagctccgtcccagacctcagtgtatttctgcgcctcatcgtacgttggtaacaccggcgaactgtttttcggtgaaggcagccgtctgacggtcctggaagatctgaaaaatgtgtttccgccggaagtcgcagtgttcgaaccgtcggaagctgaaattagccatacccagaaagcgacgctggtttgcctggccaccggtttttatccggatcatgtggaactgtcctggtgggttaacggtaaagaagtgcactcaggcgtttgtacggatccgcagccgctgaaagaacaaccggcgctgaatgactcgcgctatgccctgagctctcgtctgcgcgttagcgcgaccttctggcaggatccgcgtaaccactttcgctgtcaggtccaattctacggtctgtccgaaaatgatgaatggacccaggaccgtgcgaaaccggtcacgcaaatcgtgtcagcggaagcctggggccgcgcagat

SEQ ID NO: 9 - protein, 5 aa, Homo sapiens
GGGGS

SEQ ID NO: 10 - protein, 107 aa, Homo sapiens [sequence omitted]

SEQ ID NO: 11 - DNA, 321 bp, Homo sapiens
  source 1..321: mol_type = other DNA
gatattcagatgacgcaatccccgagttccctgtcagcttcggttggtgatcgtgtcaccattacgtgtcgcgcgagccaggacatccgtaactatctgaattggtaccagcaaaaaccgggtaaagctccgaaactgctgatttattacacctcccgtctggaatcaggtgtgccgtcgcgttttagcggctctggtagtggcaccgattataccctgacgatctcatcgctgcagccggaagactttgcgacgtattactgccagcaaggcaacaccctgccgtggacgttcggtcagggcaccaaagttgaaatcaaa

SEQ ID NO: 12 - protein, 355 aa, synthetic construct
  source 1..355: note = Amino acid sequence of fusion protein
DIQMTQSPSSLSASVGDRVTITCRASQDIRNYLNWYQQKPGKAPKLLIYYTSRLESGVPSRFSGSGSGTDYTLTISSLQPEDFATYYCQQGNTLPWTFGQGTKVEIKGGGGSNAGVTQTPKFQVLKTGQSMTLQCAQDMNHEYMSWYRQDPGMGLRLIHYSVAIQTTDQGEVPNGYNVSRSTTEDFPLRLLSAAPSQTSVYFCASSYVGNTGELFFGEGSRLTVLEDLKNVFPPEVAVFEPSEAEISHTQKATLVCLATGFYPDHVELSWWVNGKEVHSGVCTDPQPLKEQPALNDSRYALSSRLRVSATFWQDPRNHFRCQVQFYGLSENDEWTQDRAKPVTQIVSAEAWGRAD

SEQ ID NO: 13 - DNA, 1065 bp, synthetic construct
  source 1..1065: mol_type = other DNA; note = Nucleic acid sequence of fusion protein
gatattcagatgacgcaatccccgagttccctgtcagcttcggttggtgatcgtgtcaccattacgtgtcgcgcgagccaggacatccgtaactatctgaattggtaccagcaaaaaccgggtaaagctccgaaactgctgatttattacacctcccgtctggaatcaggtgtgccgtcgcgttttagcggctctggtagtggcaccgattataccctgacgatctcatcgctgcagccggaagactttgcgacgtattactgccagcaaggcaacaccctgccgtggacgttcggtcagggcaccaaagttgaaatcaaaggcggtggcggtagcaatgccggtgttacccagacgccgaaattccaagtcctgaaaaccggccagtcgatgacgctgcagtgtgcacaagatatgaatcatgaatatatgagctggtaccgccaagacccgggtatgggcctgcgtctgattcactatagcgtggccatccagaccacggatcaaggtgaagttccgaacggctacaatgtctcccgctcaaccacggaagactttccgctgcgtctgctgagcgcagcaccgtcgcagaccagcgtgtatttctgcgcaagctcttacgttggtaacaccggcgaactgtttttcggtgaaggcagccgcctgacggtcctggaagatctgaaaaatgtgtttccgccggaagtcgcggtgttcgaaccgtccgaagccgaaatttcacatacccagaaagcaacgctggtgtgcctggctaccggtttttatccggatcatgtggaactgtcttggtgggttaacggtaaagaagtgcacagtggcgtttgtacggatccgcagccgctgaaagaacaaccggcactgaatgactcccgttatgctctgagttcccgtctgcgcgtttcagccaccttctggcaggatccgcgtaaccactttcgctgtcaggtccaattctacggtctgtctgaaaatgatgaatggacccaggaccgtgcaaaaccggtcacgcaaatcgtgagtgcagaagcctggggccgcgcagat

SEQ ID NO: 14 - protein, 122 aa, synthetic construct
  source 1..122: note = Amino acid sequence of heavy chain variable region with mutation
EVQLVESGGGLVQPGGSLRLSCAASGYSFTGYTMNWVRQAPGKCLEWVALINPYKGVSTYNQKFKDRFTISVDKSKNTAYLQMNSLRAEDTAVYYCARSGYYGDSDWYFDVWGQGTLVTVSS

SEQ ID NO: 15 - DNA, 366 bp, synthetic construct
  source 1..366: mol_type = other DNA; note = Nucleic acid sequence of heavy chain variable region with mutation
gaagttcagctggtcgaaagcggtggcggtctggtccaaccgggcggttcactgcgtctgtcgtgtgcggcctctggttatagttttaccggctacacgatgaattgggttcgccaggcaccgggtaaatgcctggaatgggtcgctctgattaacccgtataaaggcgtgtctacctacaatcagaaatttaaagatcgcttcaccatcagcgtggacaaatctaaaaacacggcatatctgcaaatgaatagtctgcgtgcagaagataccgctgtgtattactgcgctcgctctggttattacggcgatagtgactggtattttgacgtttggggtcagggcaccctggtgaccgttagttcc

SEQ ID NO: 16 - protein, 108 aa, synthetic construct
  source 1..108: note = Amino acid sequence of light chain variable region with mutation
DIQMTQSPSSLSASVGDRVTITCRASQDIRNYLNWYQQKPGKAPKLLIYYTSRLESGVPSRFSGSGSGTDYTLTISSLQPEDFATYYCQQGNTLPWTFGCGTKVEIKR

SEQ ID NO: 17 - DNA, 324 bp, synthetic construct
  source 1..324: mol_type = other DNA; note = Nucleic acid sequence of light chain variable region with mutation
gatattcagatgacgcagtctccgagcagcctgtccgcctccgtgggtgaccgtgttaccattacctgtcgtgccagccaagatattcgtaactatctgaattggtaccagcaaaaaccgggtaaagccccgaaactgctgatttattacacctcgcgtctggaaagcggcgtgccgtctcgctttagtggctccggttcaggcaccgattataccctgacgatcagctctctgcagccggaagactttgcaacgtattactgccagcagggtaacaccctgccgtggacgttcggttgcggcaccaaagttgaaattaaacgt

SEQ ID NO: 18 - protein, 370 aa, synthetic construct
  source 1..370: note = Amino acid sequence of fusion protein
EVQLVESGGGLVQPGGSLRLSCAASGYSFTGYTMNWVRQAPGKCLEWVALINPYKGVSTYNQKFKDRFTISVDKSKNTAYLQMNSLRAEDTAVYYCARSGYYGDSDWYFDVWGQGTLVTVSSGGGGSNAGVTQTPKFQVLKTGQSMTLQCAQDMNHEYMSWYRQDPGMGLRLIHYSVAIQTTDQGEVPNGYNVSRSTTEDFPLRLLSAAPSQTSVYFCASSYVGNTGELFFGEGSRLTVLEDLKNVFPPEVAVFEPSEAEISHTQKATLVCLATGFYPDHVELSWWVNGKEVHSGVCTDPQPLKEQPALNDSRYALSSRLRVSATFWQDPRNHFRCQVQFYGLSENDEWTQDRAKPVTQIVSAEAWGRAD

SEQ ID NO: 19 - DNA, 1110 bp, synthetic construct
  source 1..1110: mol_type = other DNA; note = Nucleic acid sequence of fusion protein
gaagttcagctggtcgaaagcggtggcggtctggtccaaccgggcggttcactgcgtctgtcgtgtgcggcctctggttatagttttaccggctacacgatgaattgggttcgccaggcaccgggtaaatgcctggaatgggtcgctctgattaacccgtataaaggcgtgtctacctacaatcagaaatttaaagatcgcttcaccatcagcgtggacaaatctaaaaacacggcatatctgcaaatgaatagtctgcgtgcagaagataccgctgtgtattactgcgctcgctctggttattacggcgatagtgactggtattttgacgtttggggtcagggcaccctggtgaccgttagttccggcggtggcggtagcaacgcaggtgttacccagacgccgaaattccaagtcctgaaaaccggccagtctatgacgctgcagtgtgcgcaagatatgaaccatgaatacatgagttggtaccgtcaggacccgggtatgggtctgcgtctgattcactattctgtggcgatccagaccacggatcaaggtgaagttccgaacggctacaatgtctcgcgtagcaccacggaagactttccgctgcgtctgctgtccgcagctccgtcccagacctcagtgtatttctgcgcctcatcgtacgttggtaacaccggcgaactgtttttcggtgaaggcagccgtctgacggtcctggaagatctgaaaaatgtgtttccgccggaagtcgcagtgttcgaaccgtcggaagctgaaattagccatacccagaaagcgacgctggtttgcctggccaccggtttttatccggatcatgtggaactgtcctggtgggttaacggtaaagaagtgcactcaggcgtttgtacggatccgcagccgctgaaagaacaaccggcgctgaatgactcgcgctatgccctgagctctcgtctgcgcgttagcgcgaccttctggcaggatccgcgtaaccactttcgctgtcaggtccaattctacggtctgtccgaaaatgatgaatggacccaggaccgtgcgaaaccggtcacgcaaatcgtgtcagcggaagcctggggccgcgcagat

SEQ ID NO: 20 - protein, 122 aa, synthetic construct
  source 1..122: note = Amino acid sequence of heavy chain variable region with mutation
EVQLVESGGGLVQPGGSLRLSCAASGYSFTGYTMNWVRQAPGKGLEWVALINPYKGVSTYNQKFKDRFTISVDKSKNTAYLQMNSLRAEDTAVYYCARSGYYGDSDWYFDVWGCGTLVTVSS

SEQ ID NO: 21 - DNA, 366 bp, synthetic construct
  source 1..366: mol_type = other DNA; note = Nucleic acid sequence of heavy chain variable region with mutation
gaagttcagctggtcgaaagcggtggcggtctggtccaaccgggcggttcactgcgtctgtcgtgtgcggcctctggttatagttttaccggctacacgatgaattgggttcgccaggcaccgggtaaaggcctggaatgggtcgctctgattaacccgtataaaggcgtgtctacctacaatcagaaatttaaagatcgcttcaccatcagcgtggacaaatctaaaaacacggcatatctgcaaatgaatagtctgcgtgcagaagataccgctgtgtattactgcgctcgctctggttattacggcgatagtgactggtattttgacgtttggggttgcggcaccctggtgaccgttagttcc

SEQ ID NO: 22 - protein, 108 aa, synthetic construct
  source 1..108: note = Amino acid sequence of light chain variable region with mutation
DIQMTQSPSSLSASVGDRVTITCRASQDIRNYLNWYQQKPGKCPKLLIYYTSRLESGVPSRFSGSGSGTDYTLTISSLQPEDFATYYCQQGNTLPWTFGQGTKVEIKR

SEQ ID NO: 23 - DNA, 324 bp, synthetic construct
  source 1..324: mol_type = other DNA; note = Nucleic acid sequence of light chain variable region with mutation
gatattcagatgacgcagtctccgagcagcctgtccgcctccgtgggtgaccgtgttaccattacctgtcgtgccagccaagatattcgtaactatctgaattggtaccagcaaaaaccgggtaaatgcccgaaactgctgatttattacacctcgcgtctggaaagcggcgtgccgtctcgctttagtggctccggttcaggcaccgattataccctgacgatcagctctctgcagccggaagactttgcaacgtattactgccagcagggtaacaccctgccgtggacgttcggtcagggcaccaaagttgaaattaaacgt

SEQ ID NO: 24 - protein, 370 aa, synthetic construct
  source 1..370: note = Amino acid sequence of fusion protein
EVQLVESGGGLVQPGGSLRLSCAASGYSFTGYTMNWVRQAPGKGLEWVALINPYKGVSTYNQKFKDRFTISVDKSKNTAYLQMNSLRAEDTAVYYCARSGYYGDSDWYFDVWGCGTLVTVSSGGGGSNAGVTQTPKFQVLKTGQSMTLQCAQDMNHEYMSWYRQDPGMGLRLIHYSVAIQTTDQGEVPNGYNVSRSTTEDFPLRLLSAAPSQTSVYFCASSYVGNTGELFFGEGSRLTVLEDLKNVFPPEVAVFEPSEAEISHTQKATLVCLATGFYPDHVELSWWVNGKEVHSGVCTDPQPLKEQPALNDSRYALSSRLRVSATFWQDPRNHFRCQVQFYGLSENDEWTQDRAKPVTQIVSAEAWGRAD

SEQ ID NO: 25 - DNA, 1110 bp, synthetic construct
  source 1..1110: mol_type = other DNA; note = Nucleic acid sequence of fusion protein
gaagttcagctggtcgaaagcggtggcggtctggtccaaccgggcggttcactgcgtctgtcgtgtgcggcctctggttatagttttaccggctacacgatgaattgggttcgccaggcaccgggtaaaggcctggaatgggtcgctctgattaacccgtataaaggcgtgtctacctacaatcagaaatttaaagatcgcttcaccatcagcgtggacaaatctaaaaacacggcatatctgcaaatgaatagtctgcgtgcagaagataccgctgtgtattactgcgctcgctctggttattacggcgatagtgactggtattttgacgtttggggttgcggcaccctggtgaccgttagttccggcggtggcggtagcaacgcaggtgttacccagacgccgaaattccaagtcctgaaaaccggccagtctatgacgctgcagtgtgcgcaagatatgaaccatgaatacatgagttggtaccgtcaggacccgggtatgggtctgcgtctgattcactattctgtggcgatccagaccacggatcaaggtgaagttccgaacggctacaatgtctcgcgtagcaccacggaagactttccgctgcgtctgctgtccgcagctccgtcccagacctcagtgtatttctgcgcctcatcgtacgttggtaacaccggcgaactgtttttcggtgaaggcagccgtctgacggtcctggaagatctgaaaaatgtgtttccgccggaagtcgcagtgttcgaaccgtcggaagctgaaattagccatacccagaaagcgacgctggtttgcctggccaccggtttttatccggatcatgtggaactgtcctggtgggttaacggtaaagaagtgcactcaggcgtttgtacggatccgcagccgctgaaagaacaaccggcgctgaatgactcgcgctatgccctgagctctcgtctgcgcgttagcgcgaccttctggcaggatccgcgtaaccactttcgctgtcaggtccaattctacggtctgtccgaaaatgatgaatggacccaggaccgtgcgaaaccggtcacgcaaatcgtgtcagcggaagcctggggccgcgcagat

SEQ ID NO: 26 - protein, 355 aa, synthetic construct
  source 1..355: note = Amino acid sequence of fusion protein
DIQMTQSPSSLSASVGDRVTITCRASQDIRNYLNWYQQKPGKCPKLLIYYTSRLESGVPSRFSGSGSGTDYTLTISSLQPEDFATYYCQQGNTLPWTFGQGTKVEIKGGGGSNAGVTQTPKFQVLKTGQSMTLQCAQDMNHEYMSWYRQDPGMGLRLIHYSVAIQTTDQGEVPNGYNVSRSTTEDFPLRLLSAAPSQTSVYFCASSYVGNTGELFFGEGSRLTVLEDLKNVFPPEVAVFEPSEAEISHTQKATLVCLATGFYPDHVELSWWVNGKEVHSGVCTDPQPLKEQPALNDSRYALSSRLRVSATFWQDPRNHFRCQVQFYGLSENDEWTQDRAKPVTQIVSAEAWGRAD

SEQ ID NO: 27 - DNA, 1065 bp, synthetic construct
  source 1..1065: mol_type = other DNA; note = Nucleic acid sequence of fusion protein
gatattcagatgacgcagtctccgagcagcctgtccgcctccgtgggtgaccgtgttaccattacctgtcgtgccagccaagatattcgtaactatctgaattggtaccagcaaaaaccgggtaaatgcccgaaactgctgatttattacacctcgcgcctggaaagcggtgtgccgtctcgttttagcggttctggcagtggtaccgattataccctgacgatctcatcgctgcagccggaagactttgcgacgtattactgccagcagggtaacaccctgccgtggacgttcggccagggtaccaaagttgaaatcaaaggtggcggtggcagcaatgccggcgttacccagacgccgaaattccaagtcctgaaaaccggccagtctatgacgctgcagtgtgcacaagatatgaaccatgaatacatgagttggtaccgccaagacccgggcatgggtctgcgtctgattcactatagcgtggccatccagaccacggatcaaggcgaagttccgaacggttacaatgtctcccgctcaaccacggaagactttccgctgcgtctgctgagcgcagcaccgtcgcagaccagcgtgtatttctgcgcaagctcttacgttggcaacaccggtgaactgtttttcggcgaaggttctcgcctgacggtcctggaagatctgaaaaatgtgtttccgccggaagtcgcggtgttcgaaccgtcggaagccgaaattagccatacccagaaagcaacgctggtgtgcctggctaccggcttttatccggatcatgtggaactgtcctggtgggttaacggcaaagaagtgcactcaggtgtttgtacggatccgcagccgctgaaagaacaaccggcactgaatgactcgcgttatgctctgagttcccgtctgcgcgttagcgccaccttctggcaggatccgcgtaaccactttcgctgtcaggtccaattctacggcctgtccgaaaatgatgaatggacccaggaccgtgcaaaaccggtcacgcaaatcgtgtcagcagaagcctggggccgcgcagat

SEQ ID NO: 28 - protein, 355 aa, synthetic construct
  source 1..355: note = Amino acid sequence of fusion protein
  VAR_SEQ 240: note = Xaa can be any naturally occurring amino acid
DIQMTQSPSSLSASVGDRVTITCRASQDIRNYLNWYQQKPGKAPKLLIYYTSRLESGVPSRFSGSGSGTDYTLTISSLQPEDFATYYCQQGNTLPWTFGCGTKVEIKGGGGSNAGVTQTPKFQVLKTGQSMTLQCAQDMNHEYMSWYRQDPGMGLRLIHYSVAIQTTDQGEVPNGYNVSRSTTEDFPLRLLSAAPSQTSVYFCASSYVGNTGELFFGEGSRLTVLEDLKNVFPPEVAVFXPSEAEISHTQKATLVCLATGFYPDHVELSWWVNGKEVHSGVCTDPQPLKEQPALNDSRYALSSRLRVSATFWQDPRNHFRCQVQFYGLSENDEWTQDRAKPVTQIVSAEAWGRAD

SEQ ID NO: 29 - DNA, 1065 bp, synthetic construct
  source 1..1065: mol_type = other DNA; note = Nucleic acid sequence of fusion protein
gatattcagatgacgcagtctccgagcagcctgtccgcctccgtgggtgaccgtgttaccattacctgtcgtgccagccaagatattcgtaactatctgaattggtaccagcaaaaaccgggtaaagccccgaaactgctgatttattacacctcgcgtctggaaagcggcgtgccgtctcgctttagtggctccggttcaggcaccgattataccctgacgatcagctctctgcagccggaagactttgcaacgtattactgccagcagggtaacaccctgccgtggacgttcggttgcggcaccaaagttgaaatcaaaggtggcggtggcagcaatgccggcgttacccagacgccgaaattccaagtcctgaaaaccggccagtctatgacgctgcagtgtgcacaagatatgaaccatgaatacatgagttggtaccgccaagacccgggcatgggtctgcgtctgattcactatagcgtggccatccagaccacggatcaaggcgaagttccgaacggttacaatgtctcccgctcaaccacggaagactttccgctgcgtctgctgagcgcagcaccgtcgcagaccagcgtgtatttctgcgcaagctcttacgttggcaacaccggtgaactgtttttcggcgaaggttctcgcctgacggtcctggaagatctgaaaaatgtgtttccgccggaagtcgcggtgttcraaccgtcggaagccgaaattagccatacccagaaagcaacgctggtgtgcctggctaccggcttttatccggatcatgtggaactgtcctggtgggttaacggcaaagaagtgcactcaggtgtttgtacggatccgcagccgctgaaagaacaaccggcactgaatgactcgcgttatgctctgagttcccgtctgcgcgttagcgccaccttctggcaggatccgcgtaaccactttcgctgtcaggtccaattctacggcctgtccgaaaatgatgaatggacccaggaccgtgcaaaaccggtcacgcaaatcgtgtcagcagaagcctggggccgcgcagat

SEQ ID NO: 30 - protein, 205 aa, synthetic construct
  source 1..205: note = Amino acid sequence of AFP TCR alpha chain with mutation
SQQGEEDPQALSIQEGENATMNCSYKDRITNLQWYRQNSGRGLVHLILIRSNEREKHSGRLRVTLDTSKKSSSLLITASRAADTASYFCATDLEAEYKYIFGTGTRLKVLANIQNPDPAVYQLRDSKSSDKSVCLFTDFDSQTNVSQSKDSDVYITDKTVLDMRSMDFKSNSAVAWSNKSDFACANAFNNSIIPEDTFFCSPESS

SEQ ID NO: 31 - DNA, 618 bp, synthetic construct
  source 1..618: mol_type = other DNA; note = Nucleic acid sequence of AFP TCR alpha chain with mutation
agtcaacagggagaagaggatcctcaggccttgagcatccaggagggtgaaaatgccaccatgaactgcagttacaaagatcgtataaccaatttacagtggtatagacaaaattcaggtagaggccttgtccacctaattttaatacgttcaaatgaaagagagaaacacagtggaagattaagagtcacgcttgacacttccaagaaaagcagttccttgttgatcacggcttcccgggcagcagacactgcttcttacttctgtgctacggacctggaagcagaatacaaatacatctttggaacaggcaccaggctgaaggttttagcaaatatccagaacccagaccccgccgtgtatcagctgagggactccaagagctccgataagagcgtgtgcctgttcaccgactttgattctcagacaaacgtgagccagtctaaggacagcgacgtgtacatcaccgacaagacagtgctggatatgcgctccatggacttcaagagcaactccgccgtggcctggtctaataagagcgatttcgcctgcgccaacgcctttaacaattccatcatccctgaggataccttcttttgttctccagaaagttcctaa

SEQ ID NO: 32 - protein, 368 aa, synthetic construct
  source 1..368: note = Amino acid sequence of fusion protein
EVQLVESGGGLVQPGGSLRLSCAASGYSFTGYTMNWVRQAPGKGLEWVALINPYKGVSTYNQKFKDRFTISVDKSKNTAYLQMNSLRAEDTAVYYCARSGYYGDSDWYFDVWGCGTLVTVSSGGGGSETGVTQSPTHLIKTRGQQVTLRCSSQSGHNTVSWYQQALGQGPQFIFQYYRQVANGRGNFPPRFSGLQFPNYSSELNVNALELDDSALYLCASSKDAGPVFFGQGTRLTVVEDLKNVFPPEVAVFEPSECEISHTQKATLVCLATGFYPDHVELSWWVNGKEVHSGVSTDPQPLKEQPALNDSRYALSSRLRVSATFWQNPRNHFRCQVQFYGLSENDEWTQDRAKPVTQIVSAEAWGRAD

SEQ ID NO: 33 - DNA, 1107 bp, synthetic construct
  source 1..1107: mol_type = other DNA; note = Nucleic acid sequence of fusion protein
gaagttcagctggtcgaaagcggtggcggtctggtccaaccgggcggttcactgcgtctgtcgtgtgcggcctctggttatagttttaccggctacacgatgaattgggttcgccaggcaccgggtaaaggcctggaatgggtcgctctgattaacccgtataaaggcgtgtctacctacaatcagaaatttaaagatcgcttcaccatcagcgtggacaaatctaaaaacacggcatatctgcaaatgaatagtctgcgtgcagaagataccgctgtgtattactgcgctcgctctggttattacggcgatagtgactggtattttgacgtttggggttgcggcaccctggtgaccgttagttccggcggtggcggtagcgaaactggagtaacccaaagtcccacacacctgatcaaaacgagaggacagcaagtgactctgagatgctcttctcagtctgggcacaacactgtgtcctggtaccaacaggccctgggtcaggggccccagtttatctttcagtattataggcaggtggcgaatggcagaggaaacttccctcctagattctcaggtctccagttccctaattatagctctgagctgaatgtgaacgccttggagctggacgactcggccctgtatctctgtgccagcagcaaggacgcgggtccggttttctttggacaaggcaccagactcacagttgtagaggacctgaagaacgtgttcccccctgaggtggccgtgtttgagccaagcgagtgcgagatctcccacacccagaaggccaccctggtgtgcctggccacaggcttctaccccgatcacgtggagctgagctggtgggtgaacggcaaggaggtgcacagcggcgtgtccaccgacccacagcccctgaaggagcagcctgccctgaatgattctagatacgccctgtctagccggctgagagtgagcgccaccttttggcagaacccacggaatcacttcagatgtcaggtgcagttttatggcctgagcgagaacgatgagtggacccaggacagggcaaagccagtgacacagatcgtgtccgccgaggcttggggtcgtgcagattaa

SEQ ID NO: 34 - protein, 90 aa, synthetic construct
  source 1..90: note = Amino acid sequence of TRAC*01 with mutation
IQNPDPAVYQLRDSKSSDKSVCLFTDFDSQTNVSQSKDSDVYITDKTVLDMRSMDFKSNSAVAWSNKSDFACANAFNNSIIPEDTFFPSP

SEQ ID NO: 35 - protein, 128 aa, synthetic construct
  source 1..128: note = Amino acid sequence of TRBC*01 with mutation
DLNKVFPPEVAVFEPSEAEISHTQKATLVCLATGFFPDHVELSWWVNGKEVHSGVSTDPQPLKEQPALNDSRYCLSSRLRVSATFWQNPRNHFRCQVQFYGLSENDEWTQDRAKPVTQIVSAEAWGRA

SEQ ID NO: 36 - protein, 128 aa, synthetic construct
  source 1..128: note = Amino acid sequence of TRBC*02 with mutation
DLKNVFPPEVAVFEPSEAEISHTQKATLVCLATGFYPDHVELSWWVNGKEVHSGVSTDPQPLKEQPALNDSRYCLSSRLRVSATFWQNPRNHFRCQVQFYGLSENDEWTQDRAKPVTQIVSAEAWGRA

SEQ ID NO: 37 - protein, 9 aa, Homo sapiens
SLLMWITQC

SEQ ID NO: 38 - protein, 9 aa, Homo sapiens
FMNKFIYEI